European Patent Application EP 4 582 452 A1, published July 9, 2025. Title: Novel Anti-PD-L1 Chimeric Antigen Receptor and Immune Cell Expressing the Same. Applicant: KOREA RESEARCH INSTITUTE OF BIOSCIENCE AND BIOTECHNOLOGY. Application KR. The sequence listing filed with the application follows.

SEQUENCE LISTING (35 sequences)

SEQ ID NO: 1 - skipped

SEQ ID NO: 2 - protein, 17 aa, synthetic construct
XISXSGXXXYYADSVKG

SEQ ID NO: 3 - protein, 12 aa, synthetic construct
GRGRVLWTTFDH

SEQ ID NO: 4 - protein, 12 aa, synthetic construct
STVSSLQRGFDL

SEQ ID NO: 5 - protein, 10 aa, synthetic construct
RRTLVSAFDV

SEQ ID NO: 6 - protein, 10 aa, synthetic construct
RGSSRGAFDY

SEQ ID NO: 7 - protein, 12 aa, synthetic construct
DRIWYQGSGFDI

SEQ ID NO: 8 - protein, 11 aa, synthetic construct
RASQXIXXXLN

SEQ ID NO: 9 - protein, 7 aa, synthetic construct
AXSXLQS

SEQ ID NO: 10 - protein, 9 aa, synthetic construct
QQXYXXPXT

SEQ ID NO: 11 - protein, 5 aa, synthetic construct
DYEMS

SEQ ID NO: 12 - protein, 17 aa, synthetic construct
AISGSGSYTYYADSVKG

SEQ ID NO: 13 - protein, 11 aa, synthetic construct
RASQSISSWLN

SEQ ID NO: 14 - protein, 7 aa, synthetic construct
AASNLQS

SEQ ID NO: 15 - protein, 9 aa, synthetic construct
QQSYSFPWT

SEQ ID NO: 16 - protein, 5 aa, synthetic construct
DYAMS

SEQ ID NO: 17 - protein, 17 aa, synthetic construct
AISQSGGTIYYADSVKG

SEQ ID NO: 18 - protein, 11 aa, synthetic construct
RASQDISNWLN

SEQ ID NO: 19 - protein, 7 aa, synthetic construct
ATSRLQS

SEQ ID NO: 20 - protein, 9 aa, synthetic construct
QQTYSTPLT

SEQ ID NO: 21 - protein, 5 aa, synthetic construct
SYAMN

SEQ ID NO: 22 - protein, 17 aa, synthetic construct
RISSSGGYTYYADSVKG

SEQ ID NO: 23 - protein, 11 aa, synthetic construct
RASQSISNYLN

SEQ ID NO: 24 - protein, 7 aa, synthetic construct
ATSSLQS

SEQ ID NO: 25 - protein, 9 aa, synthetic construct
QQSYTFPWT

SEQ ID NO: 26 - protein, 5 aa, synthetic construct
NYGMH

SEQ ID NO: 27 - protein, 17 aa, synthetic construct
AISSSGGSTYYADSVKG

SEQ ID NO: 28 - protein, 11 aa, synthetic construct
RASQSISNWLN

SEQ ID NO: 29 - protein, 7 aa, synthetic construct
AASSLQS

SEQ ID NO: 30 - protein, 9 aa, synthetic construct
QQSYSFPWT

SEQ ID NO: 31 - protein, 5 aa, synthetic construct
DYAMH

SEQ ID NO: 32 - protein, 17 aa, synthetic construct
GISSSGSRKYYADSVKG

SEQ ID NO: 33 - protein, 11 aa, synthetic construct
RASQDIGNYLN

SEQ ID NO: 34 - protein, 7 aa, synthetic construct
AASRLQS

SEQ ID NO: 35 - protein, 9 aa, synthetic construct
QQSYSTPYT